European Patent Application EP 4 534 562 A1, published April 9, 2025. Title: BISPECIFIC ANTIBODY AND APPLICATION THEREOF. Applicant: RemeGen (Shanghai) Co., Ltd. Application CN. The sequence listing filed with the application follows.

SEQUENCE LISTING (26 sequences)

SEQ ID NO: 1 - protein, 5 aa, synthetic construct
TSTMS

SEQ ID NO: 2 - protein, 17 aa, synthetic construct
FITSAGATTNYADSVKD

SEQ ID NO: 3 - protein, 8 aa, synthetic construct
LVTLWNVY

SEQ ID NO: 4 - protein, 30 aa, synthetic construct
QVQLQESGGGLVQPGGSLRLSCAASGFTFS

SEQ ID NO: 5 - protein, 14 aa, synthetic construct
WYRQAPGKERELVA

SEQ ID NO: 6 - protein, 32 aa, synthetic construct
RFTMSRDNDKNTVYLQMNVLKPEDTAMYYCRA

SEQ ID NO: 7 - protein, 11 aa, synthetic construct
WGQGTQVTVSS

SEQ ID NO: 8 - protein, 117 aa, synthetic construct
QVQLQESGGGLVQPGGSLRLSCAASGFTFSTSTMSWYRQAPGKERELVAFITSAGATTNYADSVKDRFTMSRDNDKNTVYLQMNVLKPEDTAMYYCRALVTLWNVYWGQGTQVTVSS

SEQ ID NO: 9 - protein, 30 aa, synthetic construct
EVQLLESGGGLVQPGGSLRLSCAASGFTFS

SEQ ID NO: 10 - protein, 14 aa, synthetic construct
WYRQAPGKERELVS

SEQ ID NO: 11 - protein, 32 aa, synthetic construct
RFTMSRDNSKNTVYLQMNSLRAEDTAVYYCRA

SEQ ID NO: 12 - protein, 11 aa, synthetic construct
WGQGTLVTVSS

SEQ ID NO: 13 - protein, 117 aa, synthetic construct
EVQLLESGGGLVQPGGSLRLSCAASGFTFSTSTMSWYRQAPGKERELVSFITSAGATTYYADSVKGRFTMSRDNSKNTVYLQMNSLRAEDTAVYYCRALVTLWNVYWGQGTLVTVSS

SEQ ID NO: 14 - protein, 117 aa, synthetic construct
EVQLLESGGGLVQPGGSLRLSCAASGFTFSTSTMSWYRQAPGKERELVAFITSAGATTYYADSVKGRFTMSRDNSKNTVYLQMNSLRAEDTAVYYCRALVTLWNVYWGQGTLVTVSS

SEQ ID NO: 15 - protein, 231 aa, synthetic construct
EPKSCDKTHTCPPCPAPEAEGAPSVFLFPPKPKDTLMISRTPEVTCVVVDVSHEDPEVKFNWYVDGVEVHNAKTKPREEQYNSTYRVVSVLTVLHQDWLNGKEYKCKVSNKALPSSIEKTISKAKGQPREPQVYTLPPSREEMTKNQVSLTCLVKGFYPSDIAVEWESNGQPENNYKTTPPVLDSDGSFFLYSKLTVDKSRWQQGNVFSCSVMHEALHNHYTQKSLSLSPG

SEQ ID NO: 16 - protein, 442 aa, synthetic construct
QVQLVESGGGVVQPGRSLRLDCKASGITFSNSGMHWVRQAPGKGLEWVAVIWYDGSKRYYADSVKGRFTISRDNSKNTLFLQMNSLRAEDTAVYYCATNDDYWGQGTLVTVSSASTKGPSVFPLAPSSKSTSGGTAALGCLVKDYFPEPVTVSWNSGALTSGVHTFPAVLQSSGLYSLSSVVTVPSSSLGTQTYICNVNHKPSNTKVDKKVEPKSCDKTHTCPPCPAPEAEGAPSVFLFPPKPKDTLMISRTPEVTCVVVDVSHEDPEVKFNWYVDGVEVHNAKTKPREEQYNSTYRVVSVLTVLHQDWLNGKEYKCKVSNKALPSSIEKTISKAKGQPREPQVYTLPPSREEMTKNQVSLTCLVKGFYPSDIAVEWESNGQPENNYKTTPPVLDSDGSFFLYSKLTVDKSRWQQGNVFSCSVMHEALHNHYTQKSLSLSPG

SEQ ID NO: 17 - protein, 214 aa, synthetic construct
EIVLTQSPATLSLSPGERATLSCRASQSVSSYLAWYQQKPGQAPRLLIYDASNRATGIPARFSGSGSGTDFTLTISSLEPEDFAVYYCQQSSNWPRTFGQGTKVEIKRTVAAPSVFIFPPSDEQLKSGTASVVCLLNNFYPREAKVQWKVDNALQSGNSQESVTEQDSKDSTYSLSSTLTLSKADYEKHKVYACEVTHQGLSSPVTKSFNRGEC

SEQ ID NO: 18 - protein, 449 aa, synthetic construct
QVQLVQSGVEVKKPGASVKVSCKASGYTFTNYYMYWVRQAPGQGLEWMGGINPSNGGTNFNEKFKNRVTLTTDSSTTTAYMELKSLQFDDTAVYYCARRDYRFDMGFDYWGQGTTVTVSSASTKGPSVFPLAPSSKSTSGGTAALGCLVKDYFPEPVTVSWNSGALTSGVHTFPAVLQSSGLYSLSSVVTVPSSSLGTQTYICNVNHKPSNTKVDKKVEPKSCDKTHTCPPCPAPEAEGAPSVFLFPPKPKDTLMISRTPEVTCVVVDVSHEDPEVKFNWYVDGVEVHNAKTKPREEQYNSTYRVVSVLTVLHQDWLNGKEYKCKVSNKALPSSIEKTISKAKGQPREPQVYTLPPSREEMTKNQVSLTCLVKGFYPSDIAVEWESNGQPENNYKTTPPVLDSDGSFFLYSKLTVDKSRWQQGNVFSCSVMHEALHNHYTQKSLSLSPG

SEQ ID NO: 19 - protein, 218 aa, synthetic construct
EIVLTQSPATLSLSPGERATLSCRASKGVSTSGYSYLHWYQQKPGQAPRLLIYLASYLESGVPARFSGSGSGTDFTLTISSLEPEDFAVYYCQHSRDLPLTFGGGTKVEIKRTVAAPSVFIFPPSDEQLKSGTASVVCLLNNFYPREAKVQWKVDNALQSGNSQESVTEQDSKDSTYSLSSTLTLSKADYEKHKVYACEVTHQGLSSPVTKSFNRGEC

SEQ ID NO: 20 - protein, 559 aa, synthetic construct
QVQLVESGGGVVQPGRSLRLDCKASGITFSNSGMHWVRQAPGKGLEWVAVIWYDGSKRYYADSVKGRFTISRDNSKNTLFLQMNSLRAEDTAVYYCATNDDYWGQGTLVTVSSASTKGPSVFPLAPSSKSTSGGTAALGCLVKDYFPEPVTVSWNSGALTSGVHTFPAVLQSSGLYSLSSVVTVPSSSLGTQTYICNVNHKPSNTKVDKKVEPKSCDKTHTCPPCPAPEAEGAPSVFLFPPKPKDTLMISRTPEVTCVVVDVSHEDPEVKFNWYVDGVEVHNAKTKPREEQYNSTYRVVSVLTVLHQDWLNGKEYKCKVSNKALPSSIEKTISKAKGQPREPQVYTLPPSREEMTKNQVSLTCLVKGFYPSDIAVEWESNGQPENNYKTTPPVLDSDGSFFLYSKLTVDKSRWQQGNVFSCSVMHEALHNHYTQKSLSLSPGEVQLLESGGGLVQPGGSLRLSCAASGFTFSTSTMSWYRQAPGKERELVSFITSAGATTYYADSVKGRFTMSRDNSKNTVYLQMNSLRAEDTAVYYCRALVTLWNVYWGQGTLVTVSS

SEQ ID NO: 21 - protein, 214 aa, synthetic construct; identical to SEQ ID NO: 17

SEQ ID NO: 22 - protein, 566 aa, synthetic construct
QVQLVQSGVEVKKPGASVKVSCKASGYTFTNYYMYWVRQAPGQGLEWMGGINPSNGGTNFNEKFKNRVTLTTDSSTTTAYMELKSLQFDDTAVYYCARRDYRFDMGFDYWGQGTTVTVSSASTKGPSVFPLAPSSKSTSGGTAALGCLVKDYFPEPVTVSWNSGALTSGVHTFPAVLQSSGLYSLSSVVTVPSSSLGTQTYICNVNHKPSNTKVDKKVEPKSCDKTHTCPPCPAPEAEGAPSVFLFPPKPKDTLMISRTPEVTCVVVDVSHEDPEVKFNWYVDGVEVHNAKTKPREEQYNSTYRVVSVLTVLHQDWLNGKEYKCKVSNKALPSSIEKTISKAKGQPREPQVYTLPPSREEMTKNQVSLTCLVKGFYPSDIAVEWESNGQPENNYKTTPPVLDSDGSFFLYSKLTVDKSRWQQGNVFSCSVMHEALHNHYTQKSLSLSPGEVQLLESGGGLVQPGGSLRLSCAASGFTFSTSTMSWYRQAPGKERELVSFITSAGATTYYADSVKGRFTMSRDNSKNTVYLQMNSLRAEDTAVYYCRALVTLWNVYWGQGTLVTVSS

SEQ ID NO: 23 - protein, 218 aa, synthetic construct; identical to SEQ ID NO: 19

SEQ ID NO: 24 - protein, 17 aa, synthetic construct
FITSAGATTYYADSVKG

SEQ ID NO: 25 - protein, 717 aa, synthetic construct
EVQLVESGGGLVQPGGSLRLSCAASGYTFTNYGMNWVRQAPGKGLEWVGWINTYTGEPTYAADFKRRFTFSLDTSKSTAYLQMNSLRAEDTAVYYCAKYPHYYGSSHWYFDVWGQGTLVTVSSASTKGPSVFPLAPSSKSTSGGTAALGCLVKDYFPEPVTVSWNSGALTSGVHTFPAVLQSSGLYSLSSVVTVPSSSLGTQTYICNVNHKPSNTKVDKKVEPKSCDKTHTCPPCPAPEAAGGPSVFLFPPKPKDTLMISRTPEVTCVVVDVSHEDPEVKFNWYVDGVEVHNAKTKPREEQYNSTYRVVSVLTVLHQDWLNGKEYKCKVSNKALPAPIEKTISKAKGQPREPQVYTLPPSREEMTKNQVSLTCLVKGFYPSDIAVEWESNGQPENNYKTTPPVLDSDGSFFLYSKLTVDKSRWQQGNVFSCSVMHEALHNHYTQKSLSLSPGGGGGSGGGGSGGGGSGGGGSEVQLVESGGGLVQPGGSLRLSCAASGFAFSSYDMSWVRQAPGKGLDWVATISGGGRYTYYPDSVKGRFTISRDNSKNNLYLQMNSLRAEDTALYYCANRYGEAWFAYWGQGTLVTVSSGGGGSGGGGSGGGGSGGGGSDIQMTQSPSSMSASVGDRVTFTCRASQDINTYLSWFQQKPGKSPKTLIYRANRLVSGVPSRFSGSGSGQDYTLTISSLQPEDMATYYCLQYDEFPLTFGAGTKLELK

SEQ ID NO: 26 - protein, 214 aa, synthetic construct
DIQMTQSPSSLSASVGDRVTITCSASQDISNYLNWYQQKPGKAPKVLIYFTSSLHSGVPSRFSGSGSGTDFTLTISSLQPEDFATYYCQQYSTVPWTFGQGTKVEIKRTVAAPSVFIFPPSDEQLKSGTASVVCLLNNFYPREAKVQWKVDNALQSGNSQESVTEQDSKDSTYSLSSTLTLSKADYEKHKVYACEVTHQGLSSPVTKSFNRGEC